European Patent Specification EP 4 346 857 B1, published August 19, 2026. Title: Insulin-sensitizing agent and butyrate-producing bacterium. Applicant: Caelus Pharmaceuticals B.V. The sequence listing filed with the application follows.

SEQUENCE LISTING (4 sequences)

SEQ ID NO: 1 - DNA, 1482 bp, Anaerobutyricum soehngenii
tgatcctggctcaggatgaacgctggcggcgtgcctaacacatgcaagtcgaacgaagcaccttttaagattcttcggatgattgatcggtgactgagtggcggacgggtgagtaacgcgtgggtaacctgccctgtacagggggataacagttggaaacggctgctaataccgcataagcgcacgagaggacatcctcttgtgtgaaaaactccggtggtacaggatgggcccgcgtctgattagctggttggcagggtaacggcctaccaaggcgacgatcagtagccggtctgagaggatgaacggccacattggaactgagacacggtccaaactcctacgggaggcagcagtggggaatattgcacaatgggggaaaccctgatgcagcaacgccgcgtgagtgaagaagtatttcggtatgtaaagctctatcagcagggaagataatgacggtacctgactaagaagctccggctaaatacgtgccagcagccgcggtaatacgtatggagcaagcgttatccggatttactgggtgtaaagggtgcgtaggtggcagtgcaagtcagatgtgaaaggccggggctcaaccccggagctgcatttgaaactgcatagctagagtacaggagaggcaggcggaattcctagtgtagcggtgaaatgcgtagatattaggaggaacaccagtggcgaaggcggcctgctggactgttactgacactgaggcacgaaagcgtggggagcaaacaggattagataccctggtagtccacgccgtaaacgatgaatcctaggtgtcggggccgtataggcttcggtgccgtcgcaaacgcagtaagtattccacctggggagtacgttcgcaagaatgaaactcaaaggaattgacggggacccgcacaagcggtggagcatgtggtttaattcgaagcaacgcgaagaaccttaccaggtcttgacatccttctgaccactccgtaatgggagtcttccttcgggacagaagagacaggtggtgcatggttgtccgtcagctcgtgtcgtgagatgttgggttaagtcccgcaacgagcgcaacccctatcttcagtagccagcaggtaaggctgggcactctggagagactgccagggataacctggaggaaggtggggacgacgtcaaatcatcatgccccttatgatctgggcgacacacgtgctacaatggcggtcacaaagtgaggcaaacctgcgagggggagcaaaccacaaaaaggccgtcccagttcggactgtagtctgcaacccgactacacgaagctggaatcgctagtaatcgcgaatcagaatgtcgcggtgaatacgttcccgggtcttgtacacaccgcccgtcacaccatgggagtcggaaatgcccgaagccagtgacccaaccttttggagggarctgtcgaaggtggagccggtaactggggtgaagtcgtaacaaggg

SEQ ID NO: 2 - DNA, 1479 bp, Anaerobutyricum hallii
  misc_feature (617)..(617): n is a, c, g, or t
  misc_feature (955)..(955): n is a, c, g, or t
  misc_feature (1087)..(1087): n is a, c, g, or t
  misc_feature (1098)..(1098): n is a, c, g, or t
  misc_feature (1184)..(1185): n is a, c, g, or t
  misc_feature (1227)..(1227): n is a, c, g, or t
  misc_feature (1259)..(1259): n is a, c, g, or t
  misc_feature (1269)..(1269): n is a, c, g, or t
  misc_feature (1374)..(1375): n is a, c, g, or t
  misc_feature (1391)..(1391): n is a, c, g, or t
tttatttgagagtttgatcctggctcaggatgaacgctggcggcgtgcctaacacatgcaagtcgaacgaagcaccttaccwgattcttcggatgaaagwytggtgactgagtggcggacgggtgagtaacgcgtgggtaacctgccctgtacagggggataacagctggaaacggctgctaataccgcataagcgcacgaggagacatctccttgtgtgaaaaactccggtggtacaggatgggcccgcgtctgattagctggttggcagggtaacggcctaccaaggcaacgatcagtagccggtctgagaggatgaacggccacattggaactgagacacggtccaaactcctacgggaggcagcagtggggaatattgcacaatgggggaaaccctgatgcagcaacgccgcgtgagtgaagaagtatttcggtatgtaaagctctatcagcagggaagataatgacggtacctgactaagaagctccggctaaatacgtgccagcagccgcggtaatacgtatggagcaagcgttatccggatttactgggtgtaaagggtgcgtaggtggcagtgcaagtcagatgtgaaaggccggggctcaaccccggngctgcatttgaaactgcwyrgctagagtacaggagaggcaggcggaattcctagtgtagcggtgaaatgcgtagatattaggaggaacaccagtggcgaaggcggcctgctggactgttactgacactgaggcacgaaagcgtggggagcaaacaggattagataccctggtagtccacgccgtaaacgatgaatactaggtgtcggggccgtataggctycggtgccgccgctaacgcagtaagtattccacctggggagtacgttcgcaagaatgaaactcaaaggaattgacggggacccgcacaagcggtggagcatgtggtttaattcgaagnaacgcgaagaaccttaccaggtcttgacatccttctgaccgcaccttaatcggtgctttccttcgggacagaagagacaggtggtgcatggttgtcgtcagctcgtgtcgtgagatgttgggttaagtcccncaacgagcgcnacccctatcttcagtagccagcaggtaaggctgggcactctggagagactgccagggataacctggaggaaggtggggacgacgtnnaatcatcatgccccttatgatctgggcgacacacgtgctacnatggcggtcacagagtgaggcgaaccygcganggggagcaanccacaaaaaggccgtcccagttcggactgtagtctgcaacccgactacacgaagctggaatcgctagtaatcgcgaatcagaatgtcgcggtgaatacgttcccnngtcttgtacacaccgnccgtcacaccatgggagtcggaaatgcccgaagccagtgacccaacctttatggagggagctgtcgaaggtggagccggtaactgggg

SEQ ID NO: 3 - DNA, 1405 bp, Intestinimonas butyriciproducens
  misc_feature (666)..(668): n is a, c, g, or t
  misc_feature (696)..(698): n is a, c, g, or t
gtgcagtcgacggagcacccctgacggagttttcggacaacgaaagggaatgcttagtggcggacgggtgagtaacgcgtgagtaacctgccttggagtggggaatagcagccggaaacggctgctaataccgcatgatgtatctggatcgcatggttctggataccaaagatttattgctctgagatggactcgcgtctgattagctagttggtgaggtaacggctcaccaaggcgacgatcagtagccggactgagaggttggccggccacattgggactgagacacggcccagactcctacgggaggcagcagtggggaatattgggcaatgggcgaaagcctgacccagcaacgccgcgtgaaggaagaaggccctcgggttgtaaacttcttttgtcagggacgaagcaagtgacggtacctgacgaataagccacggctaactacgtgccagcagccgcggtaatacgtaggtggcaagcgttatccggatttactgggtgtaaagggcgtgtaggcgggagtgcaagtcagatgtgaaaactatgggctcaacccatagcctgcatttgaaactgtacttcttgagtgatggagaggcaggcggaattccctgtgtagcggtgaaatgcgtagatatagggaggaacaccagtggcgannncggcctgctggacattaactgacgctgnnncgcgaaagcgtggggagcaaacaggattagataccctggtagtccacgccgtaaacgatggatactaggtgtggggggtctgaccccctccgtgccgcagttaacacaataagtatcccacctggggagtacgatcgcaaggttgaaactcaaaggaattgacgggggcccgcacaagcggtggagtatgtggtttaattcgaagcaacgcgaagaaccttaccaggacttgacatcctactaacgaagcagagatgcataaggtgcccttcggggaaagtagagacaggtggtgcatggttgtcgtcagctcgtgtcgtgagatgttgggttaagtcccgcaacgagcgcaacccttattgttagttgctacgcaagagcactctagcgagactgccgttgacaaaacggaggaaggtggggacgacgtcaaatcatcatgccccttatgtcctgggccacacacgtactacaatggcggtcaacagagggaagcaaagccgcgaggtggagcaaatccctaaaagccgtcccagttcggattgcaggctgaaactcgcctgtatgaagtcggaatcgctagtaatcgcggatcagcatgccgcggtgaatacgttcccgggccttgtacacaccgcccgtcacaccatgagagtcgggaacacccgaagtccgtagcctaacagcaatggggcgcggccgaagga

SEQ ID NO: 4 - DNA, 1382 bp, Anaerostipes rhamnosivorans
  misc_feature (727)..(727): n is a, c, g, or t
  misc_feature (933)..(935): n is a, c, g, or t
tattttggattgaagttttcggatggatctccttaatgactgagtggcggacgggtgagtaacgcgtggggaacctgccctatacagggggataacagctggaaacggctgctaataccgcataagcgcacagaatcgcatgattcagtgtgaaaagccctggcagtataggatggtcccgcgtctgattagctggttggcggggtaacggcccaccaaggcgacgatcagtagccggcttgagagagtggacggccacattgggactgagacacggcccaaactcctacgggaggcagcagtggggaatattgcacaatgggggaaaccctgatgcagcgacgccgcgtgagtgaagaagtatttcggtatgtaaagctctatcagcagggaagaaataagacggtacctgactaagaagccccggctaactacgtgccagcagccgcggtaatacgtagggggcaagcgttatccggaattactgggtgtaaagggtgcgtaggtggcatgataagtcagaagtgaaagcccggggcttaaccccgggactgcttttgaaactgtaatgctagagtgcaggagaggtaagcggaattcctagtgtagcggtgaaatgcgtagatattaggaggaacaccagtggcgaaggcggcttactggactgtcactgacactgaggcacgaaagcgtggggagcaaacaggattagataccctggtagtcnacgccgtaaacgatgaatactaggtgtcggggccgtagaggcttcggtgccgcagcaaacgcagtaagtattccacctggggagtacgttcgcaagaatgaaactcaaaggaattgacggggacccgcacaagcggtggagcatgtggtttaattcgaagcaacgcgaagaaccttacctggtcttgacatccttctgaccggttnnnaaccgaacctttccttcgggacagaagtgacaggtggtgcatggttgtcgtcagctcgtgtcgtgagatgttgggttaagtcccgcaacgagcgcaacccctatctttagtagccagcatataaggtgggcactctagagagactgccagggataacctggaggaaggtggggacgacgtcaaatcatcatgccccttatggccagggctacacacgtgctacaatggcgtaaacaaagggaagcgaccccgcgagggcaagcaaatcccagaaataacgtctcagttcggattgtagtctgcaactcgactacatgaagctggaatcgctagtaatcgtgaatcagaatgtcacggtgaatacgttcccgggtcttgtacacaccgcccgtcacaccatgggagtcagtaacgcccgaagtcagtgacccaaccgcaaggaggaga